European Patent Specification EP 3 458 074 B1, published April 17, 2024. Title: COMPOSITIONS FOR THE DELIVERY OF TRNA AS NANOPARTICLES AND METHODS OF USE THEREWITH. Applicant: The Board of Regents of the University of Texas System. Application Unknown. The sequence listing filed with the application follows.

SEQUENCE LISTING (20 sequences)

SEQ ID NO: 1 - DNA, 76 bp, Artificial sequence
  Synthetic oligo
ggccgcgtggcctaatggataaggcgtctgacttcagatcagaagattgcaggttcgagtcctgccgcggtcgcca

SEQ ID NO: 2 - DNA, 76 bp, Artificial sequence
  Synthetic oligo
ggccgcguggccuaauggauaaggcgucugacuucagaucagaagauugcagguucgaguccugccgcggucgcca

SEQ ID NO: 3 - DNA, 75 bp, Artificial sequence
  Synthetic oligo
ggccucguggcgcaacgguagcgcgucugacuucagaucagaagguugcguguucaaaucacgucggggucacca

SEQ ID NO: 4 - DNA, 75 bp, Artificial sequence
  Synthetic oligo
gcguuggugguauagugguuagcauagcugccuucaaagcaguugacccggguucgauucccggccaacgcacca

SEQ ID NO: 5 - DNA, 85 bp, Artificial sequence
  Synthetic oligo
gcagcgauggccgagugguuaaggcguuggacuucaaauccaauggggucuccccgcgcagguucgaacccugcucgcugcgcca

SEQ ID NO: 6 - DNA, 75 bp, Artificial sequence
  Synthetic oligo
ggucccaugguguaaugguuagcacucuggacuuuaaauccagcgauccgaguucaaaucucggugggaccucca

SEQ ID NO: 7 - DNA, 76 bp, Artificial sequence
  Synthetic oligo
gcccggauagcucagucgguagagcaucagacuuuaaaucugaggguccaggguucaagucccuguucgggcgcca

SEQ ID NO: 8 - DNA, 86 bp, Artificial sequence
  Synthetic oligo
accaggauggccgagugguuaaggcguuggacuuuagauccaauggacauauguccgcguggguucgaaccccacuccugguacca

SEQ ID NO: 9 - DNA, 76 bp, Artificial sequence
  Synthetic oligo
gcccggcuagcucagucgguagagcaugggacucuaaaucccagggucguggguucgagccccacguugggcgcca

SEQ ID NO: 10 - DNA, 75 bp, Artificial sequence
  Synthetic oligo
ucccugguggucuagugguuaggauucggcgcuaucaccgccgcggcccggguucgauucccggucagggaacca

SEQ ID NO: 11 - DNA, 75 bp, Artificial sequence; identical to SEQ ID NO: 10
  Synthetic oligo

SEQ ID NO: 12 - DNA, 87 bp, Artificial sequence
  Synthetic oligo
gucaggauggccgaguggucuaaggcgccagacucuaguucuggucuccguauggaggcguggguucgaaucccacuucugacacca

SEQ ID NO: 13 - DNA, 86 bp, Artificial sequence
  Synthetic oligo
accaggauggccgagugguuaaggcguuggacuucagauccaauggacauauguccgcguggguucgaaccccacuccugguacca

SEQ ID NO: 14 - DNA, 76 bp, Artificial sequence
  Synthetic oligo
ccuucaauaguucagcugguagagcagaggacucuagguccuuagguugcugguucgauuccagcuugaaggacca

SEQ ID NO: 15 - DNA, 76 bp, Artificial sequence
  Synthetic oligo
ccuucaauaguucagcugguagagcagaggacuuuagguccuuagguugcugguucgauuccagcuugaaggacca

SEQ ID NO: 16 - DNA, 75 bp, Artificial sequence
  Synthetic oligo
ggccucguggcgcaacgguagcgcgucugacucuagaucagaagguugcguguucaaaucacgucggggucacca

SEQ ID NO: 17 - DNA, 85 bp, Artificial sequence
  Synthetic oligo
gcugugauggccgagugguuaaggcguuggacucgaaauccaauggggucuccccgcgcagguucgaauccugcucacagcgcca

SEQ ID NO: 18 - DNA, 85 bp, Artificial sequence
  Synthetic oligo
gcagcgauggccgagugguuaaggcguuggacuuuaaauccaauggggucuccccgcgcagguucgaacccugcucgcugcgcca

SEQ ID NO: 19 - RNA, 75 nt, Artificial sequence
  Synthetic oligo
gcguuggugguauaguggugagcauagcugccuucaaagcaguugacccggguucgauucccggccaacgcacca

SEQ ID NO: 20 - RNA, 75 nt, Artificial sequence
  Synthetic oligo
gcguuggugguauagugguaagcauagcugccuucaaagcaguugacccggguucgauucccggccaacgcacca